European Patent Specification EP 4 284 410 B1, published July 2, 2025. Title: COMPOSITIONS AND METHODS FOR THE TREATMENT OF GRAFT VERSUS HOST DISEASE. Applicant: VectivBio AG. The sequence listing filed with the application follows.

SEQUENCE LISTING (1 sequence)

SEQ ID NO: 1 - protein, 33 aa, Artificial Sequence
  APRAGLUTIDE
  MISC_FEATURE (10)..(10): Nle
  MISC_FEATURE (11)..(11): D-Phe
HGDGSFSDEXFTILDLLAARDFINWLIQTKITD